European Patent Application EP 4 613 854 A1, published September 10, 2025. Title: Method for the fermentative production of L-lysine using C. glutamicum strains expressing a heterologous nicotinamide nucleotide transhydrogenase PntAB and having an increased activity of a myo-inositol permease. Applicant: Evonik Operations GmbH. Application EP. The sequence listing filed with the application follows.

SEQUENCE LISTING (29 sequences)

SEQ ID NO: 1 - DNA, 1533 bp, Escherichia coli
  source 1..1533: mol_type = genomic DNA
atgcgaattggcataccaagagaacggttaaccaatgaaacccgtgttgcagcaacgccaaaaacagtggaacagctgctgaaactgggttttaccgtcgcggtagagagcggcgcgggtcaactggcaagttttgacgataaagcgtttgtgcaagcgggcgctgaaattgtagaagggaatagcgtctggcagtcagagatcattctgaaggtcaatgcgccgttagatgatgaaattgcgttactgaatcctgggacaacgctggtgagttttatctggcctgcgcagaatccggaattaatgcaaaaacttgcggaacgtaacgtgaccgtgatggcgatggactctgtgccgcgtatctcacgcgcacaatcgctggacgcactaagctcgatggcgaacatcgccggttatcgcgccattgttgaagcggcacatgaatttgggcgcttctttaccgggcaaattactgcggccgggaaagtgccaccggcaaaagtgatggtgattggtgcgggtgttgcaggtctggccgccattggcgcagcaaacagtctcggcgcgattgtgcgtgcattcgacacccgcccggaagtgaaagaacaagttcaaagtatgggcgcggaattcctcgagctggattttaaagaggaagctggcagcggcgatggctatgccaaagtgatgtcggacgcgttcatcaaagcggaaatggaactctttgccgcccaggcaaaagaggtcgatatcattgtcaccaccgcgcttattccaggcaaaccagcgccgaagctaattacccgtgaaatggttgactccatgaaggcgggcagtgtgattgtcgacctggcagcccaaaacggcggcaactgtgaatacaccgtgccgggtgaaatcttcactacggaaaatggtgtcaaagtgattggttataccgatcttccgggccgtctgccgacgcaatcctcacagctttacggcacaaacctcgttaatctgctgaaactgttgtgcaaagagaaagacggcaatatcactgttgattttgatgatgtggtgattcgcggcgtgaccgtgatccgtgcgggcgaaattacctggccggcaccgccgattcaggtatcagctcagccgcaggcggcacaaaaagcggcaccggaagtgaaaactgaggaaaaatgtacctgctcaccgtggcgtaaatacgcgttgatggcgctggcaatcattctttttggctggatggcaagcgttgcgccgaaagaattccttgggcacttcaccgttttcgcgctggcctgcgttgtcggttattacgtggtgtggaatgtatcgcacgcgctgcatacaccgttgatgtcggtcaccaacgcgatttcagggattattgttgtcggagcactgttgcagattggccagggcggctgggttagcttccttagttttatcgcggtgcttatagccagcattaatattttcggtggcttcaccgtgactcagcgcatgctgaaaatgttccgcaaaaattaa

SEQ ID NO: 2 - DNA, 1389 bp, Escherichia coli
  source 1..1389: mol_type = genomic DNA
atgtctggaggattagttacagctgcatacattgttgccgcgatcctgtttatcttcagtctggccggtctttcgaaacatgaaacgtctcgccagggtaacaacttcggtatcgccgggatggcgattgcgttaatcgcaaccatttttggaccggatacgggtaatgttggctggatcttgctggcgatggtcattggtggggcaattggtatccgtctggcgaagaaagttgaaatgaccgaaatgccagaactggtggcgatcctgcatagcttcgtgggtctggcggcagtgctggttggctttaacagctatctgcatcatgacgcgggaatggcaccgattctggtcaatattcacctgacggaagtgttcctcggtatcttcatcggggcggtaacgttcacgggttcggtggtggcgttcggcaaactgtgtggcaagatttcgtctaaaccattgatgctgccaaaccgtcacaaaatgaacctggcggctctggtcgtttccttcctgctgctgattgtatttgttcgcacggacagcgtcggcctgcaagtgctggcattgctgataatgaccgcaattgcgctggtattcggctggcatttagtcgcctccatcggtggtgcagatatgccagtggtggtgtcgatgctgaactcgtactccggctgggcggctgcggctgcgggctttatgctcagcaacgacctgctgattgtgaccggtgcgctggtcggttcttcgggggctatcctttcttacattatgtgtaaggcgatgaaccgttcctttatcagcgttattgcgggtggtttcggcaccgacggctcttctactggcgatgatcaggaagtgggtgagcaccgcgaaatcaccgcagaagagacagcggaactgctgaaaaactcccattcagtgatcattactccggggtacggcatggcagtcgcgcaggcgcaatatcctgtcgctgaaattactgagaaattgcgcgctcgtggtattaatgtgcgtttcggtatccacccggtcgcggggcgtttgcctggacatatgaacgtattgctggctgaagcaaaagtaccgtatgacatcgtgctggaaatggacgagatcaatgatgactttgctgataccgataccgtactggtgattggtgctaacgatacggttaacccggcggcgcaggatgatccgaagagtccgattgctggtatgcctgtgctggaagtgtggaaagcgcagaacgtgattgtctttaaacgttcgatgaacactggctatgctggtgtgcaaaacccgctgttcttcaaggaaaacacccacatgctgtttggtgacgccaaagccagcgtggatgcaatcctgaaagctctgtaa

SEQ ID NO: 3 - protein, 510 aa, Escherichia coli
MRIGIPRERLTNETRVAATPKTVEQLLKLGFTVAVESGAGQLASFDDKAFVQAGAEIVEGNSVWQSEIILKVNAPLDDEIALLNPGTTLVSFIWPAQNPELMQKLAERNVTVMAMDSVPRISRAQSLDALSSMANIAGYRAIVEAAHEFGRFFTGQITAAGKVPPAKVMVIGAGVAGLAAIGAANSLGAIVRAFDTRPEVKEQVQSMGAEFLELDFKEEAGSGDGYAKVMSDAFIKAEMELFAAQAKEVDIIVTTALIPGKPAPKLITREMVDSMKAGSVIVDLAAQNGGNCEYTVPGEIFTTENGVKVIGYTDLPGRLPTQSSQLYGTNLVNLLKLLCKEKDGNITVDFDDVVIRGVTVIRAGEITWPAPPIQVSAQPQAAQKAAPEVKTEEKCTCSPWRKYALMALAIILFGWMASVAPKEFLGHFTVFALACVVGYYVVWNVSHALHTPLMSVTNAISGIIVVGALLQIGQGGWVSFLSFIAVLIASINIFGGFTVTQRMLKMFRKN

SEQ ID NO: 4 - protein, 462 aa, Escherichia coli
MSGGLVTAAYIVAAILFIFSLAGLSKHETSRQGNNFGIAGMAIALIATIFGPDTGNVGWILLAMVIGGAIGIRLAKKVEMTEMPELVAILHSFVGLAAVLVGFNSYLHHDAGMAPILVNIHLTEVFLGIFIGAVTFTGSVVAFGKLCGKISSKPLMLPNRHKMNLAALVVSFLLLIVFVRTDSVGLQVLALLIMTAIALVFGWHLVASIGGADMPVVVSMLNSYSGWAAAAAGFMLSNDLLIVTGALVGSSGAILSYIMCKAMNRSFISVIAGGFGTDGSSTGDDQEVGEHREITAEETAELLKNSHSVIITPGYGMAVAQAQYPVAEITEKLRARGINVRFGIHPVAGRLPGHMNVLLAEAKVPYDIVLEMDEINDDFADTDTVLVIGANDTVNPAAQDDPKSPIAGMPVLEVWKAQNVIVFKRSMNTGYAGVQNPLFFKENTHMLFGDAKASVDAILKAL

SEQ ID NO: 5 - DNA, 1554 bp, Corynebacterium urealyticum
  source 1..1554: mol_type = genomic DNA
gtgcgtatcggtattccggttgagccgggtgagaaccagccgctggtggcagccacaccagacacggtcggcaagctcatcaagcttggctatgacgttgaagtacaggcaggtgccggcgaagacgccgcctaccctgacgccctctaccgcgaggccggcgcgagcatcgtaggcgaggaggtctgggaagcggacatcgtcacgacgctcgacaccccgcccaaggagaagcgcgacctcatgcgctccggagccaccctgatctgccgcatggctccaggccgcaacgaggagctcatcaacgagctcgccaaccgtggcatcaccgggctcgcgatggacgctgtgccgcgtatttcccgcgcacagtccatggatgtcctctcctccatggcaaacatcgccggctaccgcgcagtcatcgaggccgccaacgccttcggtcgactgttcaccggccaggtcaccgcggcaggtaaggtgccgccggcaaaggtctacgtcatcggcgctggtgtcgctggcctggccgcgatcggtaccgccaactccatgggcgcgatcgtcaaggccaccgacctgcgcgtcgaggcaggcgagcaggtcgagtccatgggggcggaattcgtcgccatccaggaagaggccgagaagtccgaggacggctacgccaaggagatgacccaagaccaggcggaactcgctgcgaagatctattcccagcagtccgccgaagccgacatcgtcatcaccaccgcaaacattccgggccgcacctcgccggtgctgctcaccgaggaagatgtcgccaacatgcgtccgggcagcgtcgtcgtcgacctggcggcagccaacggtggtaactgcgcgctgacgaagccgggcgaggtcttcgtcaccgataacggcgtgaccatcattggctacaccgacctggcgggccgcctgcctggccaggcctcccagctgttcggccagaacatcgtcaacctgttcaagctgatcacgccggagaaggacggccagcgcgtgctggacctggatgacgagatcatccgcaccatcaccgtcaccctcaatgacggccaggagacctccgtcctctggccgccaccaccggtgagcgtgtccgtcgccccgcagcagcagcccgcgcaggacacgcaggccgccgaggagccggagaagcaagccttcatgggtggccccttcgccaagatcggtctggccatcgccatcctactgggcgctgcaatcgtcctggtcagcccgctgggaatgagcggcaacttcgtcgtcctgaccctggccatcgtgctgggcttctacgtgatctccgctgtcaccccgaccctgcacaccccgttgatgtccgagacgaacgcgatttcaggaatcgtcctggtcggcgcgatcttgcaggtcaacagccccaatatcatcgttacggtcctcgcgttcctggcaatcgtcgtgtcctccgtcaacgtgttcggtggcttcgccatcacagaccgcatgctcggcatgttcgttaaggaggatgcataa

SEQ ID NO: 6 - DNA, 1488 bp, Corynebacterium urealyticum
  source 1..1488: mol_type = genomic DNA
atgactgccactctgattctttcgcaggcagcgaccggcgagaacgccacgctgctggattggctggcccggatctcgaacctggcctacatcgtggctgccgtgctcttcctcatggcactggccggcctctctaagccggagaccgcaaagcgcggtaacacgctgggcatgagcggtatggctgttgccatcgccgtggccatcttccaggccgtggttcactccaccaccgattccgatgccctggacccggtcatcaccgtcgtcctcattgccctggctatgagcctcggtgcggcctacggcatcaagcgcgcgcactccgtcgagatgactggtctgccgcagctgatcgcgctgttcaacggcatggtcggtctgggcgcggtcttcatcggctacaactccttcgtttccgagtccgccgactcgatgggtgctgccgcctacaacttccacctgggtgaggtcttcctcggcatcttcatcggtgccgtgaccttcaccggctcgatcctggctggcctgaagctctccggcaaggtcaagggcgccccgctgctgctgccggcccgtaacctgctgaacgtcgccatcctggtgatcagcctcgtgctcatggtcgtgttcatcctcgcgggtgaaggcaccaccgcctggatcgcggttggcatcatgaccgccctggcgctgttcatgggctggcacctggtcgctgccattggcggtggcgacatgccggtcgtcgtgtccatcatgaactcctactccggctgggcagctgccttcaccggtctgatgctgcagaacccgctgctgatcatcaccggtgcgctggtcggttcctccggtgcattcctctcctacgtgatgtgccaggcgatgaaccgctccttcctgaacgtcctgctgggcggcttcggcaccgacggtggcgcggtcgcggagggtgtcgacggcacccacaccgagatcgacaccgacgaggctgtcgcgatgctcaaggacgcgaagaacatcatgatcaccccgggctacggcatggctgtctcccaagcgcagtacacggtcgctgagctgacccgcaagctgcgcgaccagggtaagactgtccagttcggtatccacccggtcgccggtcgcctgcctggccacatgaacgtcctgctggctgaggcgaaggtcccttatgacatcgtcatggatatggaggagatcaacgacgacttcgacgaggtcgacgtggtcctggtcatcggcgcgaacgatacggtcaacccgagcgctgagatgccgggctccccgatcgccggcatgccggttctgaaggtgtgggaggctgagcgcgtgatcgtgctgaagcgttccatgggtgccggttactccggtgcgcagaacccgctgttcttcaacgagaacaccgacatgctgctcggtgatgcgaaggcatccatcgagaagctggccgcagggatcagcaactaa

SEQ ID NO: 7 - protein, 517 aa, Corynebacterium urealyticum
MRIGIPVEPGENQPLVAATPDTVGKLIKLGYDVEVQAGAGEDAAYPDALYREAGASIVGEEVWEADIVTTLDTPPKEKRDLMRSGATLICRMAPGRNEELINELANRGITGLAMDAVPRISRAQSMDVLSSMANIAGYRAVIEAANAFGRLFTGQVTAAGKVPPAKVYVIGAGVAGLAAIGTANSMGAIVKATDLRVEAGEQVESMGAEFVAIQEEAEKSEDGYAKEMTQDQAELAAKIYSQQSAEADIVITTANIPGRTSPVLLTEEDVANMRPGSVVVDLAAANGGNCALTKPGEVFVTDNGVTIIGYTDLAGRLPGQASQLFGQNIVNLFKLITPEKDGQRVLDLDDEIIRTITVTLNDGQETSVLWPPPPVSVSVAPQQQPAQDTQAAEEPEKQAFMGGPFAKIGLAIAILLGAAIVLVSPLGMSGNFVVLTLAIVLGFYVISAVTPTLHTPLMSETNAISGIVLVGAILQVNSPNIIVTVLAFLAIVVSSVNVFGGFAITDRMLGMFVKEDA

SEQ ID NO: 8 - protein, 495 aa, Corynebacterium urealyticum
MTATLILSQAATGENATLLDWLARISNLAYIVAAVLFLMALAGLSKPETAKRGNTLGMSGMAVAIAVAIFQAVVHSTTDSDALDPVITVVLIALAMSLGAAYGIKRAHSVEMTGLPQLIALFNGMVGLGAVFIGYNSFVSESADSMGAAAYNFHLGEVFLGIFIGAVTFTGSILAGLKLSGKVKGAPLLLPARNLLNVAILVISLVLMVVFILAGEGTTAWIAVGIMTALALFMGWHLVAAIGGGDMPVVVSIMNSYSGWAAAFTGLMLQNPLLIITGALVGSSGAFLSYVMCQAMNRSFLNVLLGGFGTDGGAVAEGVDGTHTEIDTDEAVAMLKDAKNIMITPGYGMAVSQAQYTVAELTRKLRDQGKTVQFGIHPVAGRLPGHMNVLLAEAKVPYDIVMDMEEINDDFDEVDVVLVIGANDTVNPSAEMPGSPIAGMPVLKVWEAERVIVLKRSMGAGYSGAQNPLFFNENTDMLLGDAKASIEKLAAGISN

SEQ ID NO: 9 - DNA, 4726 bp, synthetic construct
  source 1..4726: mol_type = other DNA
cccggggcttcacgggcggcgtcagttaacttcacattcacaccgttaagcctatgcgttggggtaaaaattatggcagattggtgcttaagtaatggactgttttcaccctttaaacttctagatttaaacacgaggggtttcggtagcacggtttagtaacttgtcaaaggcttgcaaatacccactgctactactctgatggcgattaagcgaactttactatgactcgaaaatttagaagactccacgatctcggatatttcatcattccgtttgttgaatttttaagtattgcggcaggatactttcttattaaaactgcagcggatgagtttggaaagcttaattttatcgggacgattctcgtagtcggaggggtcgtttccctgtttaccgggtggccacttctattcgcaagagtgaatgattttaggtgggatgcagtttaccttgtgggtggagcggtatttttagcattcctttttctggggccaaaggaaatgacagttcttggactggtggcgatgtttgctggtccgggaatgctaatagcagggttttcatatctgagtcgtcgtattattgcgtattttgtggaattgaggcggttgcaacctagtgattaagaggctgtgatcacaccatggcttgaagtaaatggagaacagcttgaagcgccacaaatgctcatacggtgtctgcaagaaagacatttgtaaagctgctggtagcccaggtaaaaaatgaaatcactgcaatgcgtggatagtcctgggaaatatgctcacagtggcggttgaatttggggggtttatttcattcactttggcttgaagtcgtgcaggtcaggggagtgttgcccgaaaacattgagaggaaaacaaaaaccgatgtttgattgggggaatcgtgtggtataatggtaggacgcagtgactgctatcacccttggcggtctcttgttgaaaggaataattactctaatgcgaatcggcatcccgcgcgaacgtctgactaatgagacccgtgtcgctgctaccccaaagaccgtcgaacagctgctgaagctcggcttcaccgttgcagtggagtccggcgccggacagctcgcgtccttcgatgacaaggctttcgtgcaggcaggcgcagagatcgttgagggcaactctgtctggcagtccgagatcattctcaaggtcaacgccccactggacgacgaaatcgcgttgctcaacccaggcaccaccctggtttccttcatctggcccgctcagaatccagagctcatgcaaaagctggcagagcgtaacgtgactgttatggccatggactctgtcccacgtatctcccgcgctcagtccctcgacgcactgtccagcatggccaacatcgctggctaccgcgcaatcgtcgaggcagcacacgagttcggccgcttctttaccggccagatcacagctgcaggaaaggtccctcctgcaaaagttatggttatcggtgcaggcgtagctggacttgcagcaatcggcgcagcaaactccctcggcgctatcgtccgtgcgtttgacactcgcccagaagttaaggaacaggtccagagcatgggcgctgaattcctggagctggacttcaaggaagaagcaggctccggcgacggctacgcaaaggtcatgtccgacgctttcatcaaggcagaaatggagctgttcgcagcacaggcaaaggaggtagacatcatcgttaccaccgcgctcatcccaggaaagccggcaccaaagctcatcacccgcgaaatggtcgacagcatgaaggcaggctccgtcatcgtcgaccttgcagcacaaaacggtggcaactgcgaatacacggttcctggtgagatcttcaccaccgaaaacggcgtgaaggtgatcggctacactgacctgccaggtcgtttgcctacccaatcctctcagctgtacggaaccaacctggtcaacctcctgaagctgctgtgcaaggaaaaggacggcaacatcaccgtcgacttcgacgatgttgtcattcgtggtgttactgtgattcgcgccggcgaaatcacctggcccgctccaccaatccaggtatctgcacagccacaggctgcccagaaggcagcaccagaggtgaagaccgaggaaaagtgcacctgctcaccatggcgcaaatacgcactcatggcactcgctatcatcctcttcggctggatggcgtccgtcgcaccaaaggagttcctgggccacttcaccgttttcgctctcgcttgcgtagttggctactacgttgtgtggaacgtttcccacgctctgcacactccactgatgtccgtcaccaacgccatctccggaatcattgttgtaggcgccctcctgcagatcggccagggcggttgggtttccttcctctccttcatcgctgtgttgatcgcctccatcaacatcttcggtggcttcacggtaacccagcgcatgctgaagatgttccgcaagaactaaggggtaacatatgtccggtggccttgttaccgcagcatacatcgtcgccgccatcctgttcatcttctctctggccggcctctccaagcacgaaacttcccgtcagggcaacaacttcggcatcgctggtatggcaatcgcactgatcgccaccatctttggaccggacaccggcaacgttggctggattctgctcgcaatggtgatcggcggcgccatcggcatccgccttgctaagaaggtcgaaatgaccgaaatgccagagctcgttgctattctccactcattcgtcggtctggctgcagttctggtaggattcaactcttacctgcaccacgatgcaggtatggcaccaatcctggtgaacatccacctcaccgaagttttcttgggcatcttcatcggcgctgttaccttcaccggctctgttgtcgcatttggtaagctgtgcggtaagatctcctccaagccactcatgctgccaaaccgccacaagatgaacctagcagcactggtcgtctcttttctccttctcatcgttttcgtgcgtaccgattccgtcggactgcaggtccttgctcttttgatcatgaccgccatcgcactcgttttcggctggcacctcgtagcctccatcggcggcgctgacatgccagttgtcgtcagcatgctgaactcctactccggctgggctgcagctgccgcaggcttcatgctgtccaacgatctccttatcgttaccggcgcgctggtgggctcctccggtgcaattctcagctacatcatgtgcaaggccatgaaccgctccttcatctccgtcatcgcaggcggcttcggaaccgatggctcctccaccggcgacgaccaggaagttggcgagcaccgcgaaatcaccgccgaagagaccgctgagcttcttaagaactcccactccgtcatcattaccccaggctacggtatggccgtcgcacaggcacagtacccagtcgccgaaatcacagaaaagcttcgcgcgcgtggcatcaacgttcgcttcggcatccacccagtcgcaggccgactcccaggacacatgaacgttctgctggcagaggctaaggtgccatacgatatcgttttggagatggacgaaattaacgacgacttcgcagacaccgataccgtactggttatcggcgcaaacgacactgtgaacccagccgcacaagacgacccaaagtcccctatcgcaggaatgccagtcctggaagtctggaaggcccagaacgtgatcgttttcaagcgaagcatgaacaccggatacgctggcgttcagaacccactattcttcaaggaaaacacccacatgctcttcggcgatgctaaggcctccgttgacgcaattctcaaggctctctaataaacaaaagcgttgcgcgtgtggcattgaaagcggtggaactacctattggatatgagtgtgcttcactcccgaattcggtgatttggaatccaaactttaaagaaaaacaccgctgcccctccacctgcgcgaagcaggggaggggcagcggctgagaaaaatctggagcgtgttatctatgcagtgtctgggtttttagtgcacctttccttttcggatgtccttgttgaaaatgacaccggaagtaacatcctcatcaatctcctccaaggtacgtccacgagtttcaggaacctgggtgtagatgaagatcaaggcaaccacaccgattccggcgaacatgaagaaggttccggttagtcctactgcttccatgatggttgggaagaacaatccgaggaacgcgtttgcgatccagaggaagaacactgagataccgattgcgaaaccgcgcattgccagcgggaagagctcagagagcataacccaggtagctacgttgaggaaggtctgcatggatcccacgaagaccacaaccagagtcaagataacgtaggggcgaagaggatcgccgactgggaatgctacggatgcgataccgatcaatacgtggctaatggtggtgagagaataaccggtaatgagggtggtacggcggttgatacgatccatcatccacagtgcgatgaatgcaccgacaactgcgatcactcctggcgccacgttggcgatcagagctgcattctcggagaaaccagcctcaatgagaacaacctggccgtagtacatgatggagtcctgcagg

SEQ ID NO: 10 - DNA, 4839 bp, synthetic construct
  source 1..4839: mol_type = other DNA
tctagagcttcacgggcggcgtcagttaacttcacattcacaccgttaagcctatgcgttggggtaaaaattatggcagattggtgcttaagtaatggactgttttcaccctttaaacttcgagatttaaacacgaggggtttcggtagcacggtttagtaacttgtcaaaggcttgcaaatacccactgctactactctgatggcgattaagcgaactttactatgactcgaaaatttagaagactccacgatctcggatatttcatcattccgtttgttgaatttttaagtattgcggcaggatactttcttattaaaactgcagcggatgagtttggaaagcttaattttatcgggacgattctcgtagtcggaggggtcgtttccctgtttaccgggtggccacttctattcgcaagagtgaatgattttaggtgggatgcagtttaccttgtgggtggagcggtatttttagcattcctttttctggggccaaaggaaatgacagttcttggactggtggcgatgtttgctggtccgggaatgctaatagcagggttttcatatctgagtcgtcgtattattgcgtattttgtggaattgaggcggttgcaacctagtgattaagaggctgtgatcacaccatggcttgaagtaaatggagaacagcttgaagcgccacaaatgctcatacggtgtctgcaagaaagacatttgtaaagctgctggtagcccaggtaaaaaatgaaatcactgcaatgcgtggatagtcctgggaaatatgctcacagtggcggttgaatttggggggtttatttcattcactttggcttgaagtcgtgcaggtcaggggagtgttgcccgaaaacattgagaggaaaacaaaaaccgatgtttgattgggggaatcgtgtggtataatggtaggacgcagtgactgctatcacccttggcggtctcttgttgaaaggaataattactctaatgcgtatcggtattccggttgagccgggtgagaaccagccgctggtggcagccacaccagacacggtcggcaagctcatcaagcttggctatgacgttgaagtacaggcaggtgccggcgaagacgccgcctaccctgacgccctctaccgcgaggccggcgcgagcatcgtaggcgaggaggtctgggaagcggacatcgtcacgacgctcgacaccccgcccaaggagaagcgcgacctcatgcgctccggagccaccctgatctgccgcatggctccaggccgcaacgaggagctcatcaacgagctcgccaaccgtggcatcaccgggctcgcgatggacgctgtgccgcgtatttcccgcgcacagtccatggatgtcctctcctccatggcaaacatcgccggctaccgcgcagtcatcgaggccgccaacgccttcggtcgactgttcaccggccaggtcaccgcggcaggtaaggtgccgccggcaaaggtctacgtcatcggcgctggtgtcgctggcctggccgcgatcggtaccgccaactccatgggcgcgatcgtcaaggccaccgacctgcgcgtcgaggcaggcgagcaggtcgagtccatgggggcggaattcgtcgccatccaggaagaggccgagaagtccgaggacggctacgccaaggagatgacccaagaccaggcggaactcgctgcgaagatctattcccagcagtccgccgaagccgacatcgtcatcaccaccgcaaacattccgggccgcacctcgccggtgctgctcaccgaggaagatgtcgccaacatgcgtccgggcagcgtcgtcgtcgacctggcggcagccaacggtggtaactgcgcgctgacgaagccgggcgaggtcttcgtcaccgataacggcgtgaccatcattggctacaccgacctggcgggccgcctgcctggccaggcctcccagctgttcggccagaacatcgtcaacctgttcaagctgatcacgccggagaaggacggccagcgcgtgctggacctggatgacgagatcatccgcaccatcaccgtcaccctcaatgacggccaggagacctccgtcctctggccgccaccaccggtgagcgtgtccgtcgccccgcagcagcagcccgcgcaggacacgcaggccgccgaggagccggagaagcaagccttcatgggtggccccttcgccaagatcggtctggccatcgccatcctactgggcgctgcaatcgtcctggtcagcccgctgggaatgagcggcaacttcgtcgtcctgaccctggccatcgtgctgggcttctacgtgatctccgctgtcaccccgaccctgcacaccccgttgatgtccgagacgaacgcgatttcaggaatcgtcctggtcggcgcgatcttgcaggtcaacagccccaatatcatcgttacggtcctcgcgttcctggcaatcgtcgtgtcctccgtcaacgtgttcggtggcttcgccatcacagaccgcatgctcggcatgttcgttaaggaggatgcataaaccatgactgccactctgattctttcgcaggcagcgaccggcgagaacgccacgctgctggattggctggcccggatctcgaacctggcctacatcgtggctgccgtgctcttcctcatggcactggccggcctctctaagccggagaccgcaaagcgcggtaacacgctgggcatgagcggtatggctgttgccatcgccgtggccatcttccaggccgtggttcactccaccaccgattccgatgccctggacccggtcatcaccgtcgtcctcattgccctggctatgagcctcggtgcggcctacggcatcaagcgcgcgcactccgtcgagatgactggtctgccgcagctgatcgcgctgttcaacggcatggtcggtctgggcgcggtcttcatcggctacaactccttcgtttccgagtccgccgactcgatgggtgctgccgcctacaacttccacctgggtgaggtcttcctcggcatcttcatcggtgccgtgaccttcaccggctcgatcctggctggcctgaagctctccggcaaggtcaagggcgccccgctgctgctgccggcccgtaacctgctgaacgtcgccatcctggtgatcagcctcgtgctcatggtcgtgttcatcctcgcgggtgaaggcaccaccgcctggatcgcggttggcatcatgaccgccctggcgctgttcatgggctggcacctggtcgctgccattggcggtggcgacatgccggtcgtcgtgtccatcatgaactcctactccggctgggcagctgccttcaccggtctgatgctgcagaacccgctgctgatcatcaccggtgcgctggtcggttcctccggtgcattcctctcctacgtgatgtgccaggcgatgaaccgctccttcctgaacgtcctgctgggcggcttcggcaccgacggtggcgcggtcgcggagggtgtcgacggcacccacaccgagatcgacaccgacgaggctgtcgcgatgctcaaggacgcgaagaacatcatgatcaccccgggctacggcatggctgtctcccaagcgcagtacacggtcgctgagctgacccgcaagctgcgcgaccagggtaagactgtccagttcggtatccacccggtcgccggtcgcctgcctggccacatgaacgtcctgctggctgaggcgaaggtcccttatgacatcgtcatggatatggaggagatcaacgacgacttcgacgaggtcgacgtggtcctggtcatcggcgcgaacgatacggtcaacccgagcgctgagatgccgggctccccgatcgccggcatgccggttctgaaggtgtgggaggctgagcgcgtgatcgtgctgaagcgttccatgggtgccggttactccggtgcgcagaacccgctgttcttcaacgagaacaccgacatgctgctcggtgatgcgaaggcatccatcgagaagctggccgcagggatcagcaactaataaacaaaagcgttgcgcgtgtggcattgaaagcggtggaactacctattggatatgagtgtgcttcactcccgaattcggtgatttggaatccaaactttaaagaaaaacaccgctgcccctccacctgcgcgaagcaggggaggggcagcggctgagaaaaatctggagcgtgttatctatgcagtgtctgggtttttagtgcacctttccttttcggatgtccttgttgaaaatgacaccggaagtaacatcctcatcaatctcctccaaggtacgtccacgagtttcaggaacctgggtgtagatgaagatcaaggcaaccacaccgattccggcgaacatgaagaaggttccggttagtcctactgcttccatgatggttgggaagaacaatccgaggaacgcgtttgcgatccagaggaagaacactgagataccgattgcgaaaccgcgcattgccagcgggaagagctcagagagcataacccaggtagctacgttgaggaaggtctgcatggatcccacgaagaccacaaccagagtcaagataacgtaggggcgaagaggatcgccgactgggaatgctacggatgcgataccgatcaatacgtggctaatggtggtgagagaataaccggtaatgagggtggtacggcggttgatacgatccatcatccacagtgcgatgaatgcaccgacaactgcgatcactcctggcgccacgttggcgatcagagctgcattctcggagaaaccagcctcaatgagaacaacctggccgtagtacatgatggagtcctgcagg

SEQ ID NO: 11 - DNA, 1527 bp, Corynebacterium glutamicum
  source 1..1527: mol_type = genomic DNA
atgacggacatcaaggccacatcaagtacatcggccactacagcaccaacagcaggccgaccagcgcgtcgacttggacaaatttccctcgtcgcctgtctcggcggacttctcttcggctatgacaccggtgtcgccaacggcgccgaaggccacatggcacaagaactcggactcaacgtgctgcagctcggcgttgtcatcagttcactggttttcgctgcagcctttggcgcgctgttcgctgggcgtatctcggacgaaatcgggcgtcgaaaagcaattatcactttgtccgtgctgttcttcctcggatcaatcctcgtcgtattctcccccgccggtgagctggggcagttctacggaccaggatttgccaccttggtcaccgggcgcatcatgttgggtctcgcggttggcggcgcctccacagtagttccggtgtacctcgctgaactcgcaccactagaaatccgcggctccctgaccggccgaaacgagcttgctatcgtcaccggccagctgcttgccttcgtgatcaacgcgcttatcgccgtcaccctacacggagttattgatggaatctggcgcatcatgttcgccgtctgtgccctccctgccgtcgccctcttcctcggcatgctgcggatgccggaatcaccacgctggctggtcaaccaggggcgttacgacgacgcccgccgcgtcatggagaccgtccgtacccctgagcgtgcgaaagccgaaatggatgaaatcatcgcggtgcactctgaaaacaatgcggcacttcctggtgttaagcagtcttcgggccaggcttcaggccaggtttctagcaagcacacccacatgtccatcggcgaagtcctcagcaacaaatggctggttcgtctgctcatcgccggcatcggtgttgcagttgcccagcagctcaccggcatcaacgccatcatgtactacggaacccgcgtcctcgaggaatccggcatgagcgcagaaatggctgtggttgccaacattgctttcggtgccgttgccgtcatcggtggactgatcgcactgcgcaacatggaccgcctggatcgccgcaccaccttcatcatcggcctgtcactgaccaccaccttccaccttttgatcgcagctgccggcactctccttccagaaggtaactccattcgaccattcgccatcatgatccttgttgttgggttcgtgctctccatgcagactttcctcaacgttgcagtgtgggtgtggctggcggaaatcttcccagtccgaatgaagggtatcggcaccggtatttcggtattctgcggttggggcatcaatggcgtcctagcgttgttcttcccagcactggtctccggcgtgggtatcaccttctccttccttatcttcgcagtcgtcggagtcattgccctggcgttcgtcaccaagtttgttcctgaaacccgtggccgctcacttgaagaactcgatcacgcagcattcaccggccagatcttcaagaaggcttaa

SEQ ID NO: 12 - protein, 508 aa, Corynebacterium glutamicum
MTDIKATSSTSATTAPTAGRPARRLGQISLVACLGGLLFGYDTGVANGAEGHMAQELGLNVLQLGVVISSLVFAAAFGALFAGRISDEIGRRKAIITLSVLFFLGSILVVFSPAGELGQFYGPGFATLVTGRIMLGLAVGGASTVVPVYLAELAPLEIRGSLTGRNELAIVTGQLLAFVINALIAVTLHGVIDGIWRIMFAVCALPAVALFLGMLRMPESPRWLVNQGRYDDARRVMETVRTPERAKAEMDEIIAVHSENNAALPGVKQSSGQASGQVSSKHTHMSIGEVLSNKWLVRLLIAGIGVAVAQQLTGINAIMYYGTRVLEESGMSAEMAVVANIAFGAVAVIGGLIALRNMDRLDRRTTFIIGLSLTTTFHLLIAAAGTLLPEGNSIRPFAIMILVVGFVLSMQTFLNVAVWVWLAEIFPVRMKGIGTGISVFCGWGINGVLALFFPALVSGVGITFSFLIFAVVGVIALAFVTKFVPETRGRSLEELDHAAFTGQIFKKA

SEQ ID NO: 13 - DNA, 1711 bp, synthetic construct
  source 1..1711: mol_type = other DNA
ccaggggcgaggtaaatcagatcaatatctgcgccctcctgccaatccagactgatgatgcggtcatcttggagggtgcaaaagaaagcggtcatgcccagctgatcgcggagccagcctaatttttcccgcaataaagttctgttaagcagggcgtcaacggcactttcgcccaggtggaggatgtttacgccaagccctaacaagccactgctggtgatgttgacgtacccgacttcctctaacgaagacgttattcgatagatcgacgacctcggctcatttaactgttttgccagctcagaatgagtatttggccctgccgaaagtgcgtctactaaaagtcctgctttggtgagtagctgaatggtttgcatatttgatccgtttttctaaaggttgtttttgattttgcccccgcatggggtgttttgtgacggctaaacaggttgtcttgggtaactatatcgacaaaaagtaacccacaacacaaaaagtcttgacaaaagcttatcttacgaacaagatgtccggtagatgatagttcgaaatcgggggcaaccccaatgaaagaatcagaatcattgaactagcgaggaaatgggactcacaccttcgtccctccttctcctaaaagcgtaggccggccaccttcccggttgttttaagtcgtttgaacaagctttacaagtgcacagggctaaatgctccaaacccttttccataactctgctttctggatcggttaagagctgcatatagcaacaattgtgacttcatcaaagataaaatcgttaacaacacagaccaaaacggtcagttaggtatggatatcagcaccttctgaacgggtacgggtataatggtgggcgtttgaaaaactcttcgccccacgaaaatgaaggagcataatgacggacatcaaggccacatcaagtacatcggccactacagcaccaacagcaggccgaccagcgcgtcgacttggacaaatttccctcgtcgcctgtctcggcggacttctcttcggctatgacaccggtgtcgccaacggcgccgaaggccacatggcacaagaactcggactcaacgtgctgcagctcggcgttgtcatcagttcactggttttcgctgcagcctttggcgcgctgttcgctgggcgtatctcggacgaaatcgggcgtcgaaaagcaattatcactttgtccgtgctgttcttcctcggatcaatcctcgtcgtattctcccccgccggtgagctggggcagttctacggaccaggatttgccaccttggtcaccgggcgcatcatgttgggtctcgcggttggcggcgcctccacagtagttccggtgtacctcgctgaactcgcaccactagaaatccgcggctccctgaccggccgaaacgagcttgctatcgtcaccggccagctgcttgccttcgtgatcaacgcgcttatcgccgtcaccctacacggagttattgatggaatctggcgcatcatgttcgccgtctgtgccctccctgccgtcgccctcttcctcggcatgctgcggatgccggaatcaccacgctggctggtcaaccaggggcgttacgacgacgcccgccgcgtcatggagaccgtccgtacccctgagcgtgcgaaagccgaaatggatgaaatcatcgcggtgcactctgaaaacaatgcggcacttcctggtgt

SEQ ID NO: 14 - DNA, 2052 bp, Corynebacterium glutamicum
  source 1..2052: mol_type = genomic DNA
atggcgtccaaactgacgacgacatcgcaacatattctggaaaaccttggtggaccagacaatattacttcgatgactcactgtgcgactcgccttcgcttccaagtgaaggatcaatccattgttgatcaacaagaaattgactccgacccatcagttcttggcgtagtaccccaaggatccaccggtatgcaggtggtgatgggtggatctgttgcaaactattaccaagaaatcctcaaacttgatggaatgaagcacttcgccgacggtgaagctacagagagttcatccaagaaggaatacggcggagtccgtggcaagtactcgtggattgactacgccttcgagttcttgtctgatactttccgaccaatcctgtgggccctgcttggtgcctcactgattattaccttgttggttcttgcggatactttcggtttgcaagacttccgcgctccaatggatgagcagcctgatacttatgtattcctgcactccatgtggcgctcggtcttctacttcctgccaattatggttggtgccaccgcagctcgaaagctcggcgcaaacgagtggattggtgcagctattccagccgcacttcttactccagaattcttggcactgggttctgccggcgataccgtcacagtctttggcctgccaatggttctgaatgactactccggacaggtattcccaccgctgattgcagcaattggtctgtactgggtggaaaagggactgaagaagatcatccctgaagcagtccaaatggtgttcgtcccattcttctccctgctgattatgatcccagcgaccgcattcctgcttggacctttcggcatcggtgttggtaacggaatttccaacctgcttgaagcgattaacaacttcagcccatttattctttccatcgttatcccattgctctacccattcttggttccacttggattgcactggccactaaacgccatcatgatccagaacatcaacaccctgggttacgacttcattcagggaccaatgggtgcctggaacttcgcctgcttcggcctggtcaccggcgtgttcttgctctccattaaggaacgaaacaaggccatgcgtcaggtttccctgggtggcatgttggctggtttgctcggcggcatttccgagccttccctctacggtgttctgctccgattcaagaagacctacttccgcctcctgccgggttgtttggcaggcggtatcgtgatgggcatcttcgacatcaaggcgtacgctttcgtgttcacctccttgcttaccatcccagcaatggacccatggttgggctacaccattggtatcgcagttgcattcttcgtttccatgttccttgttctcgcactggactaccgttccaacgaagagcgcgatgaggcacgtgcaaaggttgctgctgacaagcaggcagaagaagatctgaaggcagaagctaatgcaactcctgcagctccagtagctgctgcaggtgcgggagccggtgcaggtgcaggagccgctgctggcgctgcaaccgccgtggcagctaagccgaagctggccgctggggaagtagtggacattgtttccccactcgaaggcaaggcaattccactttctgaagtacctgacccaatctttgcagcaggcaagcttggaccaggcattgcaatccaaccaactggaaacaccgttgttgctccagcagacgctactgtcatccttgtccagaaatctggacacgcagtggcattgcgcttagatagcggagttgaaatccttgtccacgttggattggacaccgtgcaattgggcggcgaaggcttcaccgttcacgttgagcgcaggcagcaagtcaaggcgggggatccactgatcacttttgacgctgacttcattcgatccaaggatctacctttgatcaccccagttgtggtgtctaacgccgcgaaattcggtgaaattgaaggtattcctgcagatcaggcaaattcttccacgactgtgatcaaggtcaacggcaagaacgagtaa

SEQ ID NO: 15 - protein, 683 aa, Corynebacterium glutamicum
MASKLTTTSQHILENLGGPDNITSMTHCATRLRFQVKDQSIVDQQEIDSDPSVLGVVPQGSTGMQVVMGGSVANYYQEILKLDGMKHFADGEATESSSKKEYGGVRGKYSWIDYAFEFLSDTFRPILWALLGASLIITLLVLADTFGLQDFRAPMDEQPDTYVFLHSMWRSVFYFLPIMVGATAARKLGANEWIGAAIPAALLTPEFLALGSAGDTVTVFGLPMVLNDYSGQVFPPLIAAIGLYWVEKGLKKIIPEAVQMVFVPFFSLLIMIPATAFLLGPFGIGVGNGISNLLEAINNFSPFILSIVIPLLYPFLVPLGLHWPLNAIMIQNINTLGYDFIQGPMGAWNFACFGLVTGVFLLSIKERNKAMRQVSLGGMLAGLLGGISEPSLYGVLLRFKKTYFRLLPGCLAGGIVMGIFDIKAYAFVFTSLLTIPAMDPWLGYTIGIAVAFFVSMFLVLALDYRSNEERDEARAKVAADKQAEEDLKAEANATPAAPVAAAGAGAGAGAGAAAGAATAVAAKPKLAAGEVVDIVSPLEGKAIPLSEVPDPIFAAGKLGPGIAIQPTGNTVVAPADATVILVQKSGHAVALRLDSGVEILVHVGLDTVQLGGEGFTVHVERRQQVKAGDPLITFDADFIRSKDLPLITPVVVSNAAKFGEIEGIPADQANSSTTVIKVNGKNE

SEQ ID NO: 16 - DNA, 1680 bp, synthetic construct
  source 1..1680: mol_type = other DNA
gcagttggcgaagaggtcatggtcaaggtcatcgacatcgatctcgagcgtcgtcgtatctccctgtccctcaagcaggctgacgaggactacaccgaagagttcgacccatccaagtacggaatggctgactcctacgacgagcagggtaactacatcttccctgagggcttcgacgccgagaccaacgaatggctcgaaggcttcgatgagcagcgtcaggcttgggaagctcgctacgccgagtccgagcgtcgcttcaccgctcacaccgctcagatcgagcgtcgtcgtcagcaggctgaagaggcagctgccgaggctccggccggcaactactccactgattctgcagaagatgcacctgcagcagaagcagttgaagagtccgctggctccctcgcttccgatgagcagctcgctgctcttcgcgagaagctcgcaggtaactaatagttcctgcacctcttaagagggctcactgacgttgacagtgaaccctcccaaagagtttgctccgcataaacaccccgcactttttaaccttcacggtttgggaagtgcggggtgttttgttgtgaggcttggttttcgtacggtgtggttaagcttttggcgggcgcttcggcgaaaatacatgggcctacaacgccgtctaagcgtgaaactgggggatggggatacctgaaatcattcggggacgtgatgcggtggaggggtggtgcgggcataatctgacagtgtgtccgttggggggtttatttcattcactttggcttgaagtcgtgcaggtcaggggagtgttgcccgaaaacattgagaggaaaacaaaaaccgatgtttgattgggggaatcgtgtggtataatggtaggacgcagtgactgctatcacccttggcggtctcttgttgaaaggaataattactctaatggcgtccaaactgacgacgacatcgcaacatattctggaaaaccttggtggaccagacaatattacttcgatgactcactgtgcgactcgccttcgcttccaagtgaaggatcaatccattgttgatcaacaagaaattgactccgacccatcagttcttggcgtagtaccccaaggatccaccggtatgcaggtggtgatgggtggatctgttgcaaactattaccaagaaatcctcaaacttgatggaatgaagcacttcgccgacggtgaagctacagagagttcatccaagaaggaatacggcggagtccgtggcaagtactcgtggattgactacgccttcgagttcttgtctgatactttccgaccaatcctgtgggccctgcttggtgcctcactgattattaccttgttggttcttgcggatactttcggtttgcaagacttccgcgctccaatggatgagcagcctgatacttatgtattcctgcactccatgtggcgctcggtcttctacttcctgccaattatggttggtgccaccgcagctcgaaagctcggcgcaaacgagtggattggtgcagctattccagccgcacttcttactccagaattcttggcactgggttctgccggcgataccgtcacagtctttggcctgccaatggttctgaatgactactccggacaggtattcccaccgctgattgcagcaattggtctgtactgggtggaaaagggactg

SEQ ID NO: 17 - DNA, 1422 bp, Zymomonas mobilis
  source 1..1422: mol_type = genomic DNA
atgagttctgaaagtagtcagggtctagtcacgcgactagccctaatcgctgctataggcggcttgcttttcggttacgattcagcggttatcgctgcaatcggtacaccggttgatatccattttattgcccctcgtcacctgtctgctacggctgcggcttccctttctgggatggtcgttgttgctgttttggtcggttgtgttaccggttctttgctgtctggctggattggtattcgcttcggtcgtcgcggcggattgttgatgagttccatttgtttcgtcgccgccggttttggtgctgcgttaaccgaaaaattatttggaaccggtggttcggctttacaaattttttgctttttccggtttcttgccggtttaggtatcggtgtcgtttcaaccttgaccccaacctatattgctgaaattcgtccgccagacaaacgtggtcagatggtttctggtcagcagatggccattgtgacgggtgctttaaccggttatatctttacctggttactggctcatttcggttctatcgattgggttaatgccagtggttggtgctggtctccggcttcagaaggcctgatcggtattgccttcttattgctgctgttaaccgcaccggatacgccgcattggttggtgatgaagggacgtcattccgaggctagcaaaatccttgctcgtctggaaccgcaagccgatcctaatctgacgattcaaaagattaaagctggctttgataaagccatggacaaaagcagcgcaggtttgtttgcttttggtatcaccgttgtttttgccggtgtatccgttgctgccttccagcagttagtcggtattaacgccgtgctgtattatgcaccgcagatgttccagaatttaggttttggagctgatacggcattattgcagaccatctctatcggtgttgtgaacttcatcttcaccatgattgcttcccgtgttgttgaccgcttcggccgtaaacctctgcttatttggggtgctctcggtatggctgcaatgatggctgttttaggctgctgtttctggttcaaagtcggtggtgttttgcctttggcttctgtgcttctttatattgcagtctttggtatgtcatggggccctgtctgctgggttgttctgtcagaaatgttcccgagttccatcaagggcgcagctatgcctatcgctgttaccggacaatggttagctaatatcttggttaacttcctgtttaaggttgccgatggttctccagcattgaatcagactttcaaccacggtttctcctatctcgttttcgcagcattaagtatcttaggtggcttgattgttgctcgcttcgtgccggaaaccaaaggtcggagcctggatgaaatcgaggagatgtggcgctcccagaagtag

SEQ ID NO: 18 - protein, 473 aa, Zymomonas mobilis
MSSESSQGLVTRLALIAAIGGLLFGYDSAVIAAIGTPVDIHFIAPRHLSATAAASLSGMVVVAVLVGCVTGSLLSGWIGIRFGRRGGLLMSSICFVAAGFGAALTEKLFGTGGSALQIFCFFRFLAGLGIGVVSTLTPTYIAEIRPPDKRGQMVSGQQMAIVTGALTGYIFTWLLAHFGSIDWVNASGWCWSPASEGLIGIAFLLLLLTAPDTPHWLVMKGRHSEASKILARLEPQADPNLTIQKIKAGFDKAMDKSSAGLFAFGITVVFAGVSVAAFQQLVGINAVLYYAPQMFQNLGFGADTALLQTISIGVVNFIFTMIASRVVDRFGRKPLLIWGALGMAAMMAVLGCCFWFKVGGVLPLASVLLYIAVFGMSWGPVCWVVLSEMFPSSIKGAAMPIAVTGQWLANILVNFLFKVADGSPALNQTFNHGFSYLVFAALSILGGLIVARFVPETKGRSLDEIEEMWRSQK

SEQ ID NO: 19 - DNA, 3083 bp, synthetic construct
  source 1..3083: mol_type = other DNA
ccaggggcgaggtaaatcagatcaatatctgcgccctcctgccaatccagactgatgatgcggtcatcttggagggtgcaaaagaaagcggtcatgcccagctgatcgcggagccagcctaatttttcccgcaataaagttctgttaagcagggcgtcaacggcactttcgcccaggtggaggatgtttacgccaagccctaacaagccactgctggtgatgttgacgtacccgacttcctctaacgaagacgttattcgatagatcgacgacctcggctcatttaactgttttgccagctcagaatgagtatttggccctgccgaaagtgcgtctactaaaagtcctgctttggtgagtagctgaatggtttgcatatttgatccgtttttctaaaggttgtttttgattttgcccccgcatggggtgttttgtgacggctaaacaggttgtcttgggtaactatatcgacaaaaagtaacccacaacacaaaaagtcttgacaaaagcttatcttacgaacaagatgtccggtagatgatagttcgaaatcgggggcaaccccaatgaaagaatcagaatcattgaactagcgaggaaatgggactcacaccttcgtccctccttctcctaaaagcgtaggccggccaccttcccggttgttttaagtcgtttgaacaagctttacaagtgcacagggctaaatgctccaaacccttttccataactctgctttctggatcggttaagagctgcatatagcaacaattgtgacttcatcaaagataaaatcgttaacaacacagaccaaaacggtcagttaggtatggatatcagcaccttctgaacgggtacgggtataatggtgggcgtttgaaaaactcttcgccccacgaaaatgaaggagcataatgagttctgaaagtagtcagggtctagtcacgcgactagccctaatcgctgctataggcggcttgcttttcggttacgattcagcggttatcgctgcaatcggtacaccggttgatatccattttattgcccctcgtcacctgtctgctacggctgcggcttccctttctgggatggtcgttgttgctgttttggtcggttgtgttaccggttctttgctgtctggctggattggtattcgcttcggtcgtcgcggcggattgttgatgagttccatttgtttcgtcgccgccggttttggtgctgcgttaaccgaaaaattatttggaaccggtggttcggctttacaaattttttgctttttccggtttcttgccggtttaggtatcggtgtcgtttcaaccttgaccccaacctatattgctgaaattcgtccgccagacaaacgtggtcagatggtttctggtcagcagatggccattgtgacgggtgctttaaccggttatatctttacctggttactggctcatttcggttctatcgattgggttaatgccagtggttggtgctggtctccggcttcagaaggcctgatcggtattgccttcttattgctgctgttaaccgcaccggatacgccgcattggttggtgatgaagggacgtcattccgaggctagcaaaatccttgctcgtctggaaccgcaagccgatcctaatctgacgattcaaaagattaaagctggctttgataaagccatggacaaaagcagcgcaggtttgtttgcttttggtatcaccgttgtttttgccggtgtatccgttgctgccttccagcagttagtcggtattaacgccgtgctgtattatgcaccgcagatgttccagaatttaggttttggagctgatacggcattattgcagaccatctctatcggtgttgtgaacttcatcttcaccatgattgcttcccgtgttgttgaccgcttcggccgtaaacctctgcttatttggggtgctctcggtatggctgcaatgatggctgttttaggctgctgtttctggttcaaagtcggtggtgttttgcctttggcttctgtgcttctttatattgcagtctttggtatgtcatggggccctgtctgctgggttgttctgtcagaaatgttcccgagttccatcaagggcgcagctatgcctatcgctgttaccggacaatggttagctaatatcttggttaacttcctgtttaaggttgccgatggttctccagcattgaatcagactttcaaccacggtttctcctatctcgttttcgcagcattaagtatcttaggtggcttgattgttgctcgcttcgtgccggaaaccaaaggtcggagcctggatgaaatcgaggagatgtggcgctcccagaagtagaccccctccgatctctttggctagcacctaacaaaccgccacaccttttagaaagtgattctcgctgtgaacaactcactcgcattcaaccacgacaccctcccacagaaagtcatgtttggatatggcaagtccagtgcattcttaaagcaggaagttgaacgccgcggctcagccaaggtcatggtcattgcgggtgaacgagaaatgtcgatcgcccataaggtggcctcagaaattgaggtggcgatctggcacgacgaagttgtcatgcacgtgcccatcgaagtagccgaacgtgcgcgtgcagtggcaaccgacaatgagattgatctgctggtgtgtgttggcgacggatccaccataggtttggccaaagcaattgccatgaccactgccctgcccatcgtcgcgatccccaccacctacgcaggatcggaagcaaccaacgtgtggggtctgacggaagcagcgcgcaaaacaaccggtgttgatctgaaggtgctccccgaaacagtcatttacgattccgaactcaccatgtcgcttccagtggagatgtccgtggcatccggactcaacggcctggcgcactgcattgattctttgtggggacccaacgccgatcccatcaacgcagtgcttgcagccgaaggaatccgcgcactcaaccagggactgccgaaaattgttgcgaacccgcacagcatcgaaggacgcgacgaagccctctacggcgcctacctcgca

SEQ ID NO: 20 - DNA, 1395 bp, Escherichia coli
  source 1..1395: mol_type = genomic DNA
atgcctgacgctaaaaaacaggggcggtcaaacaaggcaatgacgtttttcgtctgcttccttgccgctctggcgggattactctttggcctggatatcggtgtaattgctggcgcactgccgtttattgcagatgaattccagattacttcgcacacgcaagaatgggtcgtaagctccatgatgttcggtgcggcagtcggtgcggtgggcagcggctggctctcctttaaactcgggcgcaaaaagagcctgatgatcggcgcaattttgtttgttgccggttcgctgttctctgcggctgcgccaaacgttgaagtactgattctttcccgcgttctactggggctggcggtgggtgtggcctcttataccgcaccgctgtacctctctgaaattgcgccggaaaaaattcgtggcagtatgatctcgatgtatcagttgatgatcactatcgggatcctcggtgcttatctttctgataccgccttcagctacaccggtgcatggcgctggatgctgggtgtgattatcatcccggcaattttgctgctgattggtgtcttcttcctgccagacagcccacgttggtttgccgccaaacgccgttttgttgatgccgaacgcgtgctgctacgcctgcgtgacaccagcgcggaagcgaaacgcgaactggatgaaatccgtgaaagtttgcaggttaaacagagtggctgggcgctgtttaaagagaacagcaacttccgccgcgcggtgttccttggcgtactgttgcaggtaatgcagcaattcaccgggatgaacgtcatcatgtattacgcgccgaaaatcttcgaactggcgggttataccaacactaccgagcaaatgtgggggaccgtgattgtcggcctgaccaacgtacttgccacctttatcgcaatcggccttgttgaccgctggggacgtaaaccaacgctaacgctgggcttcctggtgatggctgctggcatgggcgtactcggtacaatgatgcatatcggtattcactctccgtcggcgcagtatttcgccatcgccatgctgctgatgtttattgtcggttttgccatgagtgccggtccgctgatttgggtactgtgctccgaaattcagccgctgaaaggccgcgattttggcatcacctgctccactgccaccaactggattgccaacatgatcgttggcgcaacgttcctgaccatgctcaacacgctgggtaacgccaacaccttctgggtgtatgcggctctgaacgtactgtttatcctgctgacattgtggctggtaccggaaaccaaacacgtttcgctggaacatattgaacgtaatctgatgaaaggtcgtaaactgcgcgaaataggcgctcacgattaa

SEQ ID NO: 21 - protein, 464 aa, Escherichia coli
MPDAKKQGRSNKAMTFFVCFLAALAGLLFGLDIGVIAGALPFIADEFQITSHTQEWVVSSMMFGAAVGAVGSGWLSFKLGRKKSLMIGAILFVAGSLFSAAAPNVEVLILSRVLLGLAVGVASYTAPLYLSEIAPEKIRGSMISMYQLMITIGILGAYLSDTAFSYTGAWRWMLGVIIIPAILLLIGVFFLPDSPRWFAAKRRFVDAERVLLRLRDTSAEAKRELDEIRESLQVKQSGWALFKENSNFRRAVFLGVLLQVMQQFTGMNVIMYYAPKIFELAGYTNTTEQMWGTVIVGLTNVLATFIAIGLVDRWGRKPTLTLGFLVMAAGMGVLGTMMHIGIHSPSAQYFAIAMLLMFIVGFAMSAGPLIWVLCSEIQPLKGRDFGITCSTATNWIANMIVGATFLTMLNTLGNANTFWVYAALNVLFILLTLWLVPETKHVSLEHIERNLMKGRKLREIGAHD

SEQ ID NO: 22 - DNA, 3056 bp, synthetic construct
  source 1..3056: mol_type = other DNA
ccaggggcgaggtaaatcagatcaatatctgcgccctcctgccaatccagactgatgatgcggtcatcttggagggtgcaaaagaaagcggtcatgcccagctgatcgcggagccagcctaatttttcccgcaataaagttctgttaagcagggcgtcaacggcactttcgcccaggtggaggatgtttacgccaagccctaacaagccactgctggtgatgttgacgtacccgacttcctctaacgaagacgttattcgatagatcgacgacctcggctcatttaactgttttgccagctcagaatgagtatttggccctgccgaaagtgcgtctactaaaagtcctgctttggtgagtagctgaatggtttgcatatttgatccgtttttctaaaggttgtttttgattttgcccccgcatggggtgttttgtgacggctaaacaggttgtcttgggtaactatatcgacaaaaagtaacccacaacacaaaaagtcttgacaaaagcttatcttacgaacaagatgtccggtagatgatagttcgaaatcgggggcaaccccaatgaaagaatcagaatcattgaactagcgaggaaatgggactcacaccttcgtccctccttctcctaaaagcgtaggccggccaccttcccggttgttttaagtcgtttgaacaagctttacaagtgcacagggctaaatgctccaaacccttttccataactctgctttctggatcggttaagagctgcatatagcaacaattgtgacttcatcaaagataaaatcgttaacaacacagaccaaaacggtcagttaggtatggatatcagcaccttctgaacgggtacgggtataatggtgggcgtttgaaaaactcttcgccccacgaaaatgaaggagcataatgcctgacgctaaaaaacaggggcggtcaaacaaggcaatgacgtttttcgtctgcttccttgccgctctggcgggattactctttggcctggatatcggtgtaattgctggcgcactgccgtttattgcagatgaattccagattacttcgcacacgcaagaatgggtcgtaagctccatgatgttcggtgcggcagtcggtgcggtgggcagcggctggctctcctttaaactcgggcgcaaaaagagcctgatgatcggcgcaattttgtttgttgccggttcgctgttctctgcggctgcgccaaacgttgaagtactgattctttcccgcgttctactggggctggcggtgggtgtggcctcttataccgcaccgctgtacctctctgaaattgcgccggaaaaaattcgtggcagtatgatctcgatgtatcagttgatgatcactatcgggatcctcggtgcttatctttctgataccgccttcagctacaccggtgcatggcgctggatgctgggtgtgattatcatcccggcaattttgctgctgattggtgtcttcttcctgccagacagcccacgttggtttgccgccaaacgccgttttgttgatgccgaacgcgtgctgctacgcctgcgtgacaccagcgcggaagcgaaacgcgaactggatgaaatccgtgaaagtttgcaggttaaacagagtggctgggcgctgtttaaagagaacagcaacttccgccgcgcggtgttccttggcgtactgttgcaggtaatgcagcaattcaccgggatgaacgtcatcatgtattacgcgccgaaaatcttcgaactggcgggttataccaacactaccgagcaaatgtgggggaccgtgattgtcggcctgaccaacgtacttgccacctttatcgcaatcggccttgttgaccgctggggacgtaaaccaacgctaacgctgggcttcctggtgatggctgctggcatgggcgtactcggtacaatgatgcatatcggtattcactctccgtcggcgcagtatttcgccatcgccatgctgctgatgtttattgtcggttttgccatgagtgccggtccgctgatttgggtactgtgctccgaaattcagccgctgaaaggccgcgattttggcatcacctgctccactgccaccaactggattgccaacatgatcgttggcgcaacgttcctgaccatgctcaacacgctgggtaacgccaacaccttctgggtgtatgcggctctgaacgtactgtttatcctgctgacattgtggctggtaccggaaaccaaacacgtttcgctggaacatattgaacgtaatctgatgaaaggtcgtaaactgcgcgaaataggcgctcacgattaaaccccctccgatctctttggctagcacctaacaaaccgccacaccttttagaaagtgattctcgctgtgaacaactcactcgcattcaaccacgacaccctcccacagaaagtcatgtttggatatggcaagtccagtgcattcttaaagcaggaagttgaacgccgcggctcagccaaggtcatggtcattgcgggtgaacgagaaatgtcgatcgcccataaggtggcctcagaaattgaggtggcgatctggcacgacgaagttgtcatgcacgtgcccatcgaagtagccgaacgtgcgcgtgcagtggcaaccgacaatgagattgatctgctggtgtgtgttggcgacggatccaccataggtttggccaaagcaattgccatgaccactgccctgcccatcgtcgcgatccccaccacctacgcaggatcggaagcaaccaacgtgtggggtctgacggaagcagcgcgcaaaacaaccggtgttgatctgaaggtgctccccgaaacagtcatttacgattccgaactcaccatgtcgcttccagtggagatgtccgtggcatccggactcaacggcctggcgcactgcattgattctttgtggggacccaacgccgatcccatcaacgcagtgcttgcagccgaaggaatccgcgcactcaaccagggactgccgaaaattgttgcgaacccgcacagcatcgaaggacgcgacgaagccctctacggcgcctacctcgca

SEQ ID NO: 23 - DNA, 1857 bp, Corynebacterium glutamicum R
  source 1..1857: mol_type = genomic DNA
atggcaacgaaaacagacttcagccccttggtggctgatgttgtcaccgctttgggaggcgctgacaacgtgcgcagtgtcacgcactgtgccaccaggcttcgcttcaaaatcaaggattccgacaaggctgatatcgctaaggctggcaaaatcagtggcgtcattactgcgatcaactctggtggacagcatcaggttgtcatcggcaatgatgttccactggcgtatcaagcattgatggatgtacccggcatgcgcgccaaaggcattaaagatggcgatgcagaagtggacgatgatggcggttcagaggataagaactggctcaacaagttcatcgatctgatttctgcactgttttcaccgatcgtgtgggctttggccggtatcggtttgggtaaagctggtcttaccctggcgaccactgtaggaattttggatgcagaatcaagcacccacaccattttcaacgcgatgtttgatggcttgttttacttcttgccattcttcctcgcgataacggctgctaagcgatttaaagttaatcagttcattgctctcgcaattgtggccgcattgctgcaccccacgatggaagcgatggtcggtactgagggagttaccttcctggggctacctttgaccatgatgtcttattcttcatcagtgatccctgtggttgtgtcggtgtggttggccggatacctgcaacgctggttggaaaaggtactgcctggtgctgtccgtaacttcttcacgccactgatcgtggtgttggtgatggttccgttggtgctgtttaccatcggcccagtcaccatcggtgcagcaaatgcactgtctaatggcattgggttcctctttgaaacggttccttggttggccggtggcctcatgggtgcattctggcaggtcttcgtgatgtttggtctgcactggggactggtgccagtgatgatcaatgacattgcgacccaaggcttctcctacatgatggcgccactgatggctgcaattttcggacaggtcggtgcggctctagcagtgtggattaggtccaagaacgctgaagtgaaaaaggtagctggtcctggtgtcctttcaggattcttcgcaggtgttactgaaccaatcatttacggcgtgaaccttccactgaagtaccccttctatgcgggtgtcgtagctggtggaattggtggaatcatcatcgctgtgggtggcaacgcttttgatgccttcgtcttcccatcggtgatggctttcgcagcaacgctcagcgtgggtagcttcgtggcgcaactaattggttcgtcagctgcgcttatcttgggatttgtgttcactgtggtgatgtttcgaaaggaacaaaacgtcgataagcaagaaaccgacaccaccccaaatgtggctgcggccgcaagtggcacctacgtgccgctggcagagattcctgacaaggtgttttcctccggagccatgggcgatggatttggcatcgtgccggaaaacggtgagattgtttcaccggtggaaggccagttgattgcggtgcagaaatctgggcatgcatatggcatccgtggggataatggaattgaagttctggtgcacgtgggcattgacaccgtcaaaatggcaggtgagggattcgaaatcctcgtggcgcgtggcgatcacgtcaaagttgggcagccgctggccaaggttgatttgaatgctgttgcggaggctggtttcgatccgaccactgcggtgatcgtgactaactccaagaaactggaaggcttgaaattcactgatgttgagggacacgttggcgcaggagatgtagtgatgcgtatggaaccttaa

SEQ ID NO: 24 - protein, 618 aa, Corynebacterium glutamicum R
MATKTDFSPLVADVVTALGGADNVRSVTHCATRLRFKIKDSDKADIAKAGKISGVITAINSGGQHQVVIGNDVPLAYQALMDVPGMRAKGIKDGDAEVDDDGGSEDKNWLNKFIDLISALFSPIVWALAGIGLGKAGLTLATTVGILDAESSTHTIFNAMFDGLFYFLPFFLAITAAKRFKVNQFIALAIVAALLHPTMEAMVGTEGVTFLGLPLTMMSYSSSVIPVVVSVWLAGYLQRWLEKVLPGAVRNFFTPLIVVLVMVPLVLFTIGPVTIGAANALSNGIGFLFETVPWLAGGLMGAFWQVFVMFGLHWGLVPVMINDIATQGFSYMMAPLMAAIFGQVGAALAVWIRSKNAEVKKVAGPGVLSGFFAGVTEPIIYGVNLPLKYPFYAGVVAGGIGGIIIAVGGNAFDAFVFPSVMAFAATLSVGSFVAQLIGSSAALILGFVFTVVMFRKEQNVDKQETDTTPNVAAAASGTYVPLAEIPDKVFSSGAMGDGFGIVPENGEIVSPVEGQLIAVQKSGHAYGIRGDNGIEVLVHVGIDTVKMAGEGFEILVARGDHVKVGQPLAKVDLNAVAEAGFDPTTAVIVTNSKKLEGLKFTDVEGHVGAGDVVMRMEP

SEQ ID NO: 25 - DNA, 3518 bp, synthetic construct
  source 1..3518: mol_type = other DNA
ccaggggcgaggtaaatcagatcaatatctgcgccctcctgccaatccagactgatgatgcggtcatcttggagggtgcaaaagaaagcggtcatgcccagctgatcgcggagccagcctaatttttcccgcaataaagttctgttaagcagggcgtcaacggcactttcgcccaggtggaggatgtttacgccaagccctaacaagccactgctggtgatgttgacgtacccgacttcctctaacgaagacgttattcgatagatcgacgacctcggctcatttaactgttttgccagctcagaatgagtatttggccctgccgaaagtgcgtctactaaaagtcctgctttggtgagtagctgaatggtttgcatatttgatccgtttttctaaaggttgtttttgattttgcccccgcatggggtgttttgtgacggctaaacaggttgtcttgggtaactatatcgacaaaaagtaacccacaacacaaaaagtcttgacaaaagcttatcttacgaacaagatgtccggtagatgatagttcgaaatcgggggcaaccccaatgaaagaatcagaatcattgaactagcgaggaaatgggactcacaccttcgtccctccttctcctaaaagcgtaggccggccaccttcccggttgttttaagtcgtttgaacaagctttacaagtgcacagggctaaatgctccaaacccttttccataactctgctttctggatcggttaagagctgcatatagcaacaattgtgacttcatcaaagataaaatcgttaacaacacagaccaaaacggtcagttaggtatggatatcagcaccttctgaacgggtacgggtataatggtgggcgtttgaaaaactcttcgccccacgaaaatgaaggagcataatggcaacgaaaacagacttcagccccttggtggctgatgttgtcaccgctttgggaggcgctgacaacgtgcgcagtgtcacgcactgtgccaccaggcttcgcttcaaaatcaaggattccgacaaggctgatatcgctaaggctggcaaaatcagtggcgtcattactgcgatcaactctggtggacagcatcaggttgtcatcggcaatgatgttccactggcgtatcaagcattgatggatgtacccggcatgcgcgccaaaggcattaaagatggcgatgcagaagtggacgatgatggcggttcagaggataagaactggctcaacaagttcatcgatctgatttctgcactgttttcaccgatcgtgtgggctttggccggtatcggtttgggtaaagctggtcttaccctggcgaccactgtaggaattttggatgcagaatcaagcacccacaccattttcaacgcgatgtttgatggcttgttttacttcttgccattcttcctcgcgataacggctgctaagcgatttaaagttaatcagttcattgctctcgcaattgtggccgcattgctgcaccccacgatggaagcgatggtcggtactgagggagttaccttcctggggctacctttgaccatgatgtcttattcttcatcagtgatccctgtggttgtgtcggtgtggttggccggatacctgcaacgctggttggaaaaggtactgcctggtgctgtccgtaacttcttcacgccactgatcgtggtgttggtgatggttccgttggtgctgtttaccatcggcccagtcaccatcggtgcagcaaatgcactgtctaatggcattgggttcctctttgaaacggttccttggttggccggtggcctcatgggtgcattctggcaggtcttcgtgatgtttggtctgcactggggactggtgccagtgatgatcaatgacattgcgacccaaggcttctcctacatgatggcgccactgatggctgcaattttcggacaggtcggtgcggctctagcagtgtggattaggtccaagaacgctgaagtgaaaaaggtagctggtcctggtgtcctttcaggattcttcgcaggtgttactgaaccaatcatttacggcgtgaaccttccactgaagtaccccttctatgcgggtgtcgtagctggtggaattggtggaatcatcatcgctgtgggtggcaacgcttttgatgccttcgtcttcccatcggtgatggctttcgcagcaacgctcagcgtgggtagcttcgtggcgcaactaattggttcgtcagctgcgcttatcttgggatttgtgttcactgtggtgatgtttcgaaaggaacaaaacgtcgataagcaagaaaccgacaccaccccaaatgtggctgcggccgcaagtggcacctacgtgccgctggcagagattcctgacaaggtgttttcctccggagccatgggcgatggatttggcatcgtgccggaaaacggtgagattgtttcaccggtggaaggccagttgattgcggtgcagaaatctgggcatgcatatggcatccgtggggataatggaattgaagttctggtgcacgtgggcattgacaccgtcaaaatggcaggtgagggattcgaaatcctcgtggcgcgtggcgatcacgtcaaagttgggcagccgctggccaaggttgatttgaatgctgttgcggaggctggtttcgatccgaccactgcggtgatcgtgactaactccaagaaactggaaggcttgaaattcactgatgttgagggacacgttggcgcaggagatgtagtgatgcgtatggaaccttaaaccccctccgatctctttggctagcacctaacaaaccgccacaccttttagaaagtgattctcgctgtgaacaactcactcgcattcaaccacgacaccctcccacagaaagtcatgtttggatatggcaagtccagtgcattcttaaagcaggaagttgaacgccgcggctcagccaaggtcatggtcattgcgggtgaacgagaaatgtcgatcgcccataaggtggcctcagaaattgaggtggcgatctggcacgacgaagttgtcatgcacgtgcccatcgaagtagccgaacgtgcgcgtgcagtggcaaccgacaatgagattgatctgctggtgtgtgttggcgacggatccaccataggtttggccaaagcaattgccatgaccactgccctgcccatcgtcgcgatccccaccacctacgcaggatcggaagcaaccaacgtgtggggtctgacggaagcagcgcgcaaaacaaccggtgttgatctgaaggtgctccccgaaacagtcatttacgattccgaactcaccatgtcgcttccagtggagatgtccgtggcatccggactcaacggcctggcgcactgcattgattctttgtggggacccaacgccgatcccatcaacgcagtgcttgcagccgaaggaatccgcgcactcaaccagggactgccgaaaattgttgcgaacccgcacagcatcgaaggacgcgacgaagccctctacggcgcctacctcgca

SEQ ID NO: 26 - DNA, 1266 bp, Corynebacterium glutamicum
  source 1..1266: mol_type = genomic DNA; note = Exchange of nucleobase cytosine (c) at position 932 of lysC gene sequence derived from ATCC13032 wildtype to give thymine (t). The acc codon for threonine is altered to the atc codon for isoleucine.
gtggccctggtcgtacagaaatatggcggttcctcgcttgagagtgcggaacgcattagaaacgtcgctgaacggatcgttgccaccaagaaggctggaaatgatgtcgtggttgtctgctccgcaatgggagacaccacggatgaacttctagaacttgcagcggcagtgaatcccgttccgccagctcgtgaaatggatatgctcctgactgctggtgagcgtatttctaacgctctcgtcgccatggctattgagtcccttggcgcagaagcccaatctttcacgggctctcaggctggtgtgctcaccaccgagcgccacggaaacgcacgcattgttgatgtcactccaggtcgtgtgcgtgaagcactcgatgagggcaagatctgcattgttgctggtttccagggtgttaataaagaaacccgcgatgtcaccacgttgggtcgtggtggttctgacaccactgcagttgcgttggcagctgctttgaacgctgatgtgtgtgagatttactcggacgttgacggtgtgtataccgctgacccgcgcatcgttcctaatgcacagaagctggaaaagctcagcttcgaagaaatgctggaacttgctgctgttggctccaagattttggtgctgcgcagtgttgaatacgctcgtgcattcaatgtgccacttcgcgtacgctcgtcttatagtaatgatcccggcactttgattgccggctctatggaggatattcctgtggaagaagcagtccttaccggtgtcgcaaccgacaagtccgaagccaaagtaaccgttctgggtatttccgataagccaggcgaggctgcgaaggttttccgtgcgttggctgatgcagaaatcaacattgacatggttctgcagaacgtctcttctgtagaagacggcaccaccgacatcatcttcacctgccctcgttccgacggccgccgcgcgatggagatcttgaagaagcttcaggttcagggcaactggaccaatgtgctttacgacgaccaggtcggcaaagtctccctcgtgggtgctggcatgaagtctcacccaggtgttaccgcagagttcatggaagctctgcgcgatgtcaacgtgaacatcgaattgatttccacctctgagattcgtatttccgtgctgatccgtgaagatgatctggatgctgctgcacgtgcattgcatgagcagttccagctgggcggcgaagacgaagccgtcgtttatgcaggcaccggacgctaa

SEQ ID NO: 27 - protein, 421 aa, Corynebacterium glutamicum
MALVVQKYGGSSLESAERIRNVAERIVATKKAGNDVVVVCSAMGDTTDELLELAAAVNPVPPAREMDMLLTAGERISNALVAMAIESLGAEAQSFTGSQAGVLTTERHGNARIVDVTPGRVREALDEGKICIVAGFQGVNKETRDVTTLGRGGSDTTAVALAAALNADVCEIYSDVDGVYTADPRIVPNAQKLEKLSFEEMLELAAVGSKILVLRSVEYARAFNVPLRVRSSYSNDPGTLIAGSMEDIPVEEAVLTGVATDKSEAKVTVLGISDKPGEAAKVFRALADAEINIDMVLQNVSSVEDGTTDIIFTCPRSDGRRAMEILKKLQVQGNWTNVLYDDQVGKVSLVGAGMKSHPGVTAEFMEALRDVNVNIELISTSEIRISVLIREDDLDAAARALHEQFQLGGEDEAVVYAGTGR

SEQ ID NO: 28 - DNA, 1476 bp, Corynebacterium glutamicum
  source 1..1476: mol_type = genomic DNA
atggctagtaccttcattcaggccgacagccctgaaaaaagtaagaagctgcccccactcacagaaggtccgtatagaaagcggctattctacgttgcactagttgcgacgtttggtgggctgctcttcggatatgacaccggagtaatcaacggtgcactcaacccaatgacacgtgagctcggactaaccgcgttcaccgagggtgttgtaacttcttccctgctgtttggtgcagcagctggtgcgatgtttttcggtcgcatttccgacaactggggtcgccggaaaacaatcatctcacttgcagtagctttctttgtcggcaccatgatctgcgtgtttgctccatcttttgcagtaatggttgtcggacgtgtgcttcttggactcgcagttggtggcgcttccactgttgtccctgtctacctggctgaacttgctccttttgaaatccgtggctcactggctggccgtaatgagttgatgattgttgttggtcagctcgcagcttttgtcatcaatgcgattattggaaatgtttttggacaccacgatggtgtgtggcgctacatgctggcaattgccgcaatcccagcaattgccctcttctttggaatgctccgagttccagaatccccacgctggcttgttgagcgaggacgcattgatgaggctcgcgcagttcttgaaaccattcgccctctagaacgtgcccatgcagaagttgctgatgttgaacacctagcaagagaagagcacgccgtttccgagaagtccatgggcttaagggaaattttgtccagcaagtggcttgtgcgcatcctcctggtaggtatcggattgggtgtcgcacagcagctgaccggcatcaactccatcatgtactacggccaggttgttctcattgaggctggtttctccgagaatgcagctctgatcgccaacgtggcgccaggagtgatcgcagttgtcggtgcattcatcgcactgtggatgatggatcgtatcaaccgccgtaccaccctcattaccggttattctctcaccaccattagccacgtattgatcggtatcgcatccgtagcattcccagtcggcgatcctcttcgcccctacgttatcttgactctggttgtggtcttcgtgggatccatgcagaccttcctcaacgtagctacctgggttatgctctctgagctcttcccgctggcaatgcgcggtttcgcaatcggtatctcagtgttcttcctctggatcgcaaacgcgttcctcggattgttcttcccaaccatcatggaagcagtaggactaaccggaaccttcttcatgttcgccggaatcggtgtggttgccttgatcttcatctacacccaggttcctgaaactcgtggacgtaccttggaggagattgatgaggatgttacttccggtgtcattttcaacaaggacatccgaaaaggaaaggtgcactaa

SEQ ID NO: 29 - protein, 491 aa, Corynebacterium glutamicum
MASTFIQADSPEKSKKLPPLTEGPYRKRLFYVALVATFGGLLFGYDTGVINGALNPMTRELGLTAFTEGVVTSSLLFGAAAGAMFFGRISDNWGRRKTIISLAVAFFVGTMICVFAPSFAVMVVGRVLLGLAVGGASTVVPVYLAELAPFEIRGSLAGRNELMIVVGQLAAFVINAIIGNVFGHHDGVWRYMLAIAAIPAIALFFGMLRVPESPRWLVERGRIDEARAVLETIRPLERAHAEVADVEHLAREEHAVSEKSMGLREILSSKWLVRILLVGIGLGVAQQLTGINSIMYYGQVVLIEAGFSENAALIANVAPGVIAVVGAFIALWMMDRINRRTTLITGYSLTTISHVLIGIASVAFPVGDPLRPYVILTLVVVFVGSMQTFLNVATWVMLSELFPLAMRGFAIGISVFFLWIANAFLGLFFPTIMEAVGLTGTFFMFAGIGVVALIFIYTQVPETRGRTLEEIDEDVTSGVIFNKDIRKGKVH